European Patent Application EP 4 253 564 A1, published October 4, 2023. Title: Method and Kits for Amplifying Target Nucleic Acid with High Specificity. Applicant: PANAGENE INC. The sequence listing filed with the application follows.

SEQUENCE LISTING (22 sequences)

SEQ ID NO: 1 - DNA, 24 bp, Artificial Sequence
  PT 1
gtcgtccgtgttttgatttctctg

SEQ ID NO: 2 - DNA, 25 bp, Artificial Sequence
  SP 1
gcttgctctgataggaaaatgagat

SEQ ID NO: 3 - DNA, 25 bp, Artificial Sequence
  GP 1
ggacccactccatcgcacggacgac

SEQ ID NO: 4 - DNA, 15 bp, Artificial Sequence
  DP 1
ggtgattttggtcta

SEQ ID NO: 5 - DNA, 18 bp, Artificial Sequence
  PT 2
gcgtgtccaggagcttgt

SEQ ID NO: 6 - DNA, 23 bp, Artificial Sequence
  SP 2
tgtatcaaagaatggtcctgcac

SEQ ID NO: 7 - DNA, 24 bp, Artificial Sequence
  GP 2
cttgtggtagttggctggacacgc

SEQ ID NO: 8 - DNA, 12 bp, Artificial Sequence
  DP 2
gtcaaggcactc

SEQ ID NO: 9 - DNA, 23 bp, Artificial Sequence
  PT 3
gtcgtccgtgtttacggtagttt

SEQ ID NO: 10 - DNA, 22 bp, Artificial Sequence
  PT 4
gtcgtccgtgttttgtagccta

SEQ ID NO: 11 - DNA, 23 bp, Artificial Sequence
  PT 5
gtcgtccgtgttttctcggaagt

SEQ ID NO: 12 - DNA, 23 bp, Artificial Sequence
  PT 6
gtcgtccgtgttttctcggttgt

SEQ ID NO: 13 - DNA, 23 bp, Artificial Sequence
  PT 7
gtcgtccgtgttttctcgctagt

SEQ ID NO: 14 - DNA, 23 bp, Artificial Sequence
  PT 8
gtcgtccgtgttttctcgttagt

SEQ ID NO: 15 - DNA, 21 bp, Artificial Sequence
  SP 3
ccatgatagccgtctttaaca

SEQ ID NO: 16 - DNA, 25 bp, Artificial Sequence
  GP 3
cttctggaaaagtagcacggacgac

SEQ ID NO: 17 - DNA, 11 bp, Artificial Sequence
  DP 3
tacgatgcaag

SEQ ID NO: 18 - DNA, 19 bp, Artificial Sequence
  PT 9
gtcgtccgtgccttccaca

SEQ ID NO: 19 - DNA, 24 bp, Artificial Sequence
  SP 4
tgtagggcatttctgatgtgactc

SEQ ID NO: 20 - DNA, 24 bp, Artificial Sequence
  GP 4
acttgtggtagttgctggacacgc

SEQ ID NO: 21 - DNA, 25 bp, Artificial Sequence
  GP 5
agtgtcatcttgcctcacggacgac

SEQ ID NO: 22 - DNA, 13 bp, Artificial Sequence
  DP 4
cagcagtaaatct